European Patent Specification EP 3 592 155 B1, published May 6, 2026. Title: Method of reducing contamination with Chlostridium. Applicant: Nomad Bioscience GmbH UAB Nomads. The sequence listing filed with the application follows.

SEQUENCE LISTING (6 sequences)

SEQ ID NO: 1 - protein, 342 aa, Clostridium phage SM101
MQSRNNNNLKGIDVSNWKGNINFESVKNDGVEVVYIKATEGNYFKDKYAKQNYEGAKEQGLSVGFYHFFRANKGAKDQANFFIDYLNEIGAVNYDCKLALDIETTEGVGVRDLTSMCIEFLEEVKRLTGKEVVVYTYTSFANNNLDSRLGNYPVWIAHYGVNTPGANNIWSSWVGFQYSENGSVAGVNGGCDMNEFTEEIFIDSSNFNLDNATTKNVSTKLNIRAKGTTNSKIIGSIPAGETFKIKWVDEDYLGWYYVEYNGVVGYVNADYVEKLQMATTYNVSTFLNVREEGSLNSRIVDKINSGDIFRIDWVDSDFIGWYRITTKNGKVGFVNAEFVKKL

SEQ ID NO: 2 - protein, 335 aa, Clostridium perfringens CPE str. F4969
MLKGIDVSEHQGRIDWERVKGNIDFAILRAGYGRNNIDKQFIRNIEECNRLCIPVGIYWFSYAWNEEMAKNEARYVLEAIKGYRVDYPISYDLEYDTLNYASKNGVTIGKRLATDMVKAFCDEINRNGYRAMNYTNQDFLLNKFYMNELTNYPLWYAWYNSKLNRDCAIWQYSENGQVPGIPGSSVDMNYCYEDFLKKDFTLENATTCNVDTELNIRAKGTTGATIVGSIPAGDRFRIKWVDSDYLGWYYIEYQGITGYVSQDYVEKLQMATTCNVDSVLNVRAEGNTSSNIVATINPGEVFRIDWVDSDFIGWYRITTANGANGFVKSDFVKKL

SEQ ID NO: 3 - protein, 351 aa, Clostridium perfringens CPE str. F4969
MQSRSDSNFKGIDISNWQKGINLNQLKERGYDVCYIKITEGKGYVDPCFEENYNKAIAAGMKVGVYHYWRGTSSAIEQANNIVRTLGNKHIDCKIAIDVEQTDGLSYGELNNSVLQLAEELERLIGAEVCIYCNTNYARNVLDSRLGKYSLWVAHYGVNKPGDNPIWDKWAGFQYSENGTSNVNGSLDLDEFTEEIFINKESSKVTENKLFSTNARALVALDPRDNPSDNYNDLGEIYEGERIQVLAEVCDKEDYLPVKYWKDSEGRESGKVWIRSKQDYMMIDTYHRVFNVITQLDARYEPSSDSATMGYVKNGERLYVHRTEGNYSLCTYFAGNGYKTAWFTAKYLERI

SEQ ID NO: 4 - protein, 377 aa, Clostridium perfringens vB_CpeS-CP51
MYINQSNIKFNGLRYGNDPNKIIIHNADATSCSVYDIDRWHKGNGWSGIGYDYFIRKEGSVWTGRPENAIGAHTIGQNSSSIGICLEGAFMREKPTRAQLNSLYELIADIRARRGNLPVYGHKDFNNTDCPGINFPLEQFKNNSYRPTGGEIVSDNGFYRSDEERTNATIVGEGNIEVLDKNCKVIENRYISSLDRVFVLGIYPASKYIEIIYPAGNEKYHAYISIENYSRISFDYHMQYKNDNGVTYVWWDSEDVNVKEHNEELQANQKASPMYRVGKWLRVTFYRTDGTPSDGFVRYEGEQAVKFYEEEKIKEGIVKVNTYLNVRDSINGNIIGKVFNGEEVSIIWTKDGWYYIDYNTNHGKKRGYVSSKYVEEV

SEQ ID NO: 5 - protein, 212 aa, Clostridium perfringens CP26F
MIIGSRYGHSENCRGAKGLRDEVDAMKPLHFEFKKIMEQYGHTIIDCCSNANTQNGELSEGARKANAQILDLFISWHGNKGGGQGCEAWIANNSRAKPYAERMCKNFSSLGFKNRGVKYSDKYYEMRNINAPNIIFETLFLDSEKDISIWSPIPYEVMARYLANAIDPNIPLEKEQDYYRVCVQRFTNKEDAEKAQQRISNELGYYCFAEKI

SEQ ID NO: 6 - protein, 213 aa, Clostridium perfringens CP39-O
MKIALRGGHSPNCKGANVLRDEQSCMWALADEVEKVLTSHGHTVVRCETTLSNEREDVRQGAKKGYNCDMFISLHMNASDGRGNGTEAWVARSARSSIKEIASRLCKNYATLGLQNRGVKEKNYWEMTDTNCPNIIFETMFCDDKHDIDIWASTSWDKLARLIANAIDPNIPLEKEQDYYRVCVQRFTNKEDAEKAQQRISNELGYYCFAEKI